European Patent Application EP 4 471 424 A2, published December 4, 2024. Title: Adeno-Associated Virus Virions with Variant Capsid and Methods of Use Thereof. Applicant: The Regents of the University of California. Application EP Divisional of European Patent Application no. 21201945.9, filed April 20, 2012. The sequence listing filed with the application follows.

SEQUENCE LISTING (64 sequences)

SEQ ID NO: 1 - protein, 733 aa, Adeno-associated virus-2
MAADGYLPDWLEDTLSEGIRQWWKLKPGPPPPKPAERHKDDSRGLVLPGYKYLGPFNGLDKGEPVNEADAAALEHDKAYDRQLDSGDNPYLKYNHADAEFQERLKEDTSFGGNLGRAVFQAKKRVLEPLGLVEEPVKTAPGKKRPVEHSPVEPDSSSGTGKAGQQPARKRLNFGQTGDADSVPDPQPLGQPPAAPSGLGTNTMATGSGAPMADNNEGADGVGNSSGNWHCDSTWMGDRVITTSTRTWALPTYNNHLYKQISSQSGASNDNHYFGYSTPWGYFDFNRFHCHFSPRDWQRLINNNWGFRPKRLNFKLFNIQVKEVTQNDGTTTIANNLTSTVQVFTDSEYQLPYVLGSAHQGCLPPFPADVFMVPQYGYLTLNNGSQAVGRSSFYCLEYFPSQMLRTGNNFTFSYTFEDVPFHSSYAHSQSLDRLMNPLIDQYLYYLSRTNTPSGTTTQSRLQFSQAGASDIRDQSRNWLPGPCYRQQRVSKTSADNNNSEYSWTGATKYHLNGRDSLVNPGPAMASHKDDEEKFFPQSGVLIFGKQGSEKTNVDIEKVMITDEEEIRTTNPVATEQYGSVSTNLQRGNRQAATADVNTQGVLPGMVWQDRDVYLQGPIWAKIPHTDGHFHPSPLMGGFGLKHPPPQILIKNTPVPANPSTTFSAAKFASFITQYSTGQVSVEIEWELQKENSKRWNPEIQYTSNYNKSVNVDFTVDTNGVYSEPRPIGTRYLTR

SEQ ID NO: 2 - protein, 42 aa, Adeno-associated virus-2
PVATEQYGSVSTNLQRGNRQAATADVNTQGVLPGMVWQDRDV

SEQ ID NO: 3 - protein, 42 aa, Adeno-associated virus-AAV-1
PVATERFGTVAVNFQSSSTDPATGDVHAMGALPGMVWQDRDV

SEQ ID NO: 4 - protein, 42 aa, Adeno-associated virus-5
RVAYNVGGQMATNNQSSTTAPATGTYNLQEIVPGSVWMERDV

SEQ ID NO: 5 - protein, 42 aa, Adeno-associated virus-AAV-6
PVATERFGTVAVNLQSSSTDPATGDVHVMGALPGMVWQDRDV

SEQ ID NO: 6 - protein, 42 aa, Adeno-associated virus-AAV-
PVATEEYGIVSSNLQAANTAAQTQVVNNQGALPGMVWQNRDV

SEQ ID NO: 7 - protein, 42 aa, Adeno-associated virus-AAV-8
PVATEEYGIVADNLQQQNTAPQIGTVNSQGALPGMVWQNRDV

SEQ ID NO: 8 - protein, 42 aa, Adeno-associated virus-AAV-9
PVATESYGQVATNHQSAQAQAQTGWVQNQGILPGMVWQDRDV

SEQ ID NO: 9 - protein, 42 aa, Adeno-associated virus-AAV-10
PVATEQYGVVADNLQQANTGPIVGNVNSQGALPGMVWQNRDV

SEQ ID NO: 10 - protein, 224 aa, Homo sapiens
MSRKIEGFLLLLLFGYEATLGLSSTEDEGEDPWYQKACKCDCQGGPNALWSAGATSLDCIPECPYHKPLGFESGEVTPDQITCSNPEQYVGWYSSWTANKARLNSQGFGCAWLSKFQDSSQWLQIDLKEIKVISGILTQGRCDIDEWMTKYSVQYRTDERLNWIYYKDQTGNNRVFYGNSDRTSTVQNLLRPPIISRFIRLIPLGWHVRIAIRMELLECVSKCA

SEQ ID NO: 11 - protein, 247 aa, Homo sapiens
MTILFLTMVISYFGCMKAAPMKEANIRGQGGLAYPGVRTHGTLESVNGPKAGSRGLTSLADTFEHVIEELLDEDHKVRPNEENNKDADLYTSRVMLSSQVPLEPPLLFLLEEYKNYLDAANMSMMVLRHSDPARRGELSVCDSISEWVTAADKKTAVDMSGGTVTVLEKVPVSKGQLKQYFYETKCNPMGYTKEGCRGIDKRHWNSQCRTTQSYVRALTMDSKKRIGWRFIRIDTSCVCTLTIKRGR

SEQ ID NO: 12 - protein, 533 aa, Homo sapiens
MSIQVEHPAGGYKKLFETVEELSSPLTAHVTGRIPLWLTGSLLRCGPGLFEVGSEPFYHLFDGQALLHKFDFKEGHVTYHRRFIRTDAYVRAMTEKRIVITEFGTCAFPDPCKNIFSRFFSYFRGVEVTDNALVNVYPVGEDYYACTETNFITKINPETLETIKQVDLCNYVSVNGATAHPHIENDGTVYNIGNCFGKNFSIAYNIVKIPPLQADKEDPISKSEIVVQFPCSDRFKPSYVHSFGLTPNYIVFVETPVKINLFKFLSSWSLWGANYMDCFESNETMGVWLHIADKKRKKYLNNKYRTSPFNLFHHINTYEDNGFLIVDLCCWKGFEFVYNYLYLANLRENWEEVKKNARKAPQPEVRRYVLPLNIDKADTGKNLVTLPNTTATAILCSDETIWLEPEVLFSGPRQAFEFPQINYQKYCGKPYTYAYGLGLNHFVPDRLCKLNVKTKETWVWQEPDSYPSEPIFVSHPDALEEDDGVVLSVVVSPGAGQKPAYLLILNAKDLSEVARAEVEINIPVTFHGLFKKS

SEQ ID NO: 13 - protein, 7 aa, synthetic construct
  REGION 1..7: note = Synthetic peptide
LGETTRP

SEQ ID NO: 14 - protein, 7 aa, synthetic construct
  REGION 1..7: note = Synthetic peptide
NETITRP

SEQ ID NO: 15 - protein, 7 aa, synthetic construct
  REGION 1..7: note = Synthetic peptide
KAGQANN

SEQ ID NO: 16 - protein, 7 aa, synthetic construct
  REGION 1..7: note = Synthetic peptide
KDPKTTN

SEQ ID NO: 17 - RNA, 27 nt, synthetic construct
  misc_feature 1..27: note = Synthetic oligonucleotide
  source 1..27: mol_type = other RNA
cgcaatcagtgaatgcttatacatccg

SEQ ID NO: 18 - DNA, 5541 bp, synthetic construct
  misc_feature 1..5541: note = Synthetic construct
  source 1..5541: mol_type = other DNA
agcttggatccaatcaacctctggattacaaaatttgtgaaagattgactggtattcttaactatgttgctccttttacgctatgtggatacgctgctttaatgcctttgtatcatgctattgcttcccgtatggctttcattttctcctccttgtataaatcctggttgctgtctctttatgaggagttgtggcccgttgtcaggcaacgtggcgtggtgtgcactgtgtttgctgacgcaacccccactggttggggcattgccaccacctgtcagctcctttccgggactttcgctttccccctccctattgccacggcggaactcatcgccgcctgccttgcccgctgctggacaggggctcggctgttgggcactgacaattccgtggtgttgtcggggaagctgacgtcctttccatggctgctcgcctgtgttgccacctggattctgcgcgggacgtccttctgctacgtcccttcggccctcaatccagcggaccttccttcccgcggcctgctgccggctctgcggcctcttccgcgtcttcgagatctgcctcgactgtgccttctagttgccagccatctgttgtttgcccctcccccgtgccttccttgaccctggaaggtgccactcccactgtcctttcctaataaaatgaggaaattgcatcgcattgtctgagtaggtgtcattctattctggggggtggggtggggcaggacagcaagggggaggattgggaagacaatagcaggcatgctggggactcgagttaagggcgaattcccgattaggatcttcctagagcatggctacgtagataagtagcatggcgggttaatcattaactacaaggaacccctagtgatggagttggccactccctctctgcgcgctcgctcgctcactgaggccgggcgaccaaaggtcgcccgacgcccgggctttgcccgggcggcctcagtgagcgagcgagcgcgcagccttaattaacctaattcactggccgtcgttttacaacgtcgtgactgggaaaaccctggcgttacccaacttaatcgccttgcagcacatccccctttcgccagctggcgtaatagcgaagaggcccgcaccgatcgcccttcccaacagttgcgcagcctgaatggcgaatgggacgcgccctgtagcggcgcattaagcgcggcgggtgtggtggttacgcgcagcgtgaccgctacacttgccagcgccctagcgcccgctcctttcgctttcttcccttcctttctcgccacgttcgccggctttccccgtcaagctctaaatcgggggctccctttagggttccgatttagtgctttacggcacctcgaccccaaaaaacttgattagggtgatggttcacgtagtgggccatcgccccgatagacggtttttcgccctttgacgctggagttcacgttcctcaatagtggactcttgttccaaactggaacaacactcaaccctatctcggtctattcttttgatttataagggatttttccgatttcggcctattggttaaaaaatgagctgatttaacaaaaatttaacgcgaattttaacaaaatattaacgtttataatttcaggtggcatctttcggggaaatgtgcgcggaacccctatttgtttatttttctaaatacattcaaatatgtatccgctcatgagacaataaccctgataaatgcttcaataatattgaaaaaggaagagtatgagtattcaacatttccgtgtcgcccttattcccttttttgcggcattttgccttcctgtttttgctcacccagaaacgctggtgaaagtaaaagatgctgaagatcagttgggtgcacgagtgggttacatcgaactggatctcaatagtggtaagatccttgagagttttcgccccgaagaacgttttccaatgatgagcacttttaaagttctgctatgtggcgcggtattatcccgtattgacgccgggcaagagcaactcggtcgccgcatacactattctcagaatgacttggttgagtactcaccagtcacagaaaagcatcttacggatggcatgacagtaagagaattatgcagtgctgccataaccatgagtgataacactgcggccaacttacttctgacaacgatcggaggaccgaaggagctaaccgcttttttgcacaacatgggggatcatgtaactcgccttgatcgttgggaaccggagctgaatgaagccataccaaacgacgagcgtgacaccacgatgcctgtagtaatggtaacaacgttgcgcaaactattaactggcgaactacttactctagcttcccggcaacaattaatagactggatggaggcggataaagttgcaggaccacttctgcgctcggcccttccggctggctggtttattgctgataaatctggagccggtgagcgtgggtctcgcggtatcattgcagcactggggccagatggtaagccctcccgtatcgtagttatctacacgacggggagtcaggcaactatggatgaacgaaatagacagatcgctgagataggtgcctcactgattaagcattggtaactgtcagaccaagtttactcatatatactttagattgatttaaaacttcatttttaatttaaaaggatctaggtgaagatcctttttgataatctcatgaccaaaatcccttaacgtgagttttcgttccactgagcgtcagaccccgtagaaaagatcaaaggatcttcttgagatcctttttttctgcgcgtaatctgctgcttgcaaacaaaaaaaccaccgctaccagcggtggtttgtttgccggatcaagagctaccaactctttttccgaaggtaactggcttcagcagagcgcagataccaaatactgtccttctagtgtagccgtagttaggccaccacttcaagaactctgtagcaccgcctacatacctcgctctgctaatcctgttaccagtggctgctgccagtggcgataagtcgtgtcttaccgggttggactcaagacgatagttaccggataaggcgcagcggtcgggctgaacggggggttcgtgcacacagcccagcttggagcgaacgacctacaccgaactgagatacctacagcgtgagctatgagaaagcgccacgcttcccgaagggagaaaggcggacaggtatccggtaagcggcagggtcggaacaggagagcgcacgagggagcttccagggggaaacgcctggtatctttatagtcctgtcgggtttcgccacctctgacttgagcgtcgatttttgtgatgctcgtcaggggggcggagcctatggaaaaacgccagcaacgcggcctttttacggttcctggccttttgctgcggttttgctcacatgttctttcctgcgttatcccctgattctgtggataaccgtattaccgcctttgagtgagctgataccgctcgccgcagccgaacgaccgagcgcagcgagtcagtgagcgaggaagcggaagagcgcccaatacgcaaaccgcctctccccgcgcgttggccgattcattaatgcagctggcacgacaggtttcccgactggaaagcgggcagtgagcgcaacgcaattaatgtgagttagctcactcattaggcaccccaggctttacactttatgcttccggctcgtatgttgtgtggaattgtgagcggataacaatttcacacaggaaacagctatgaccatgattacgccagatttaattaaggctgcgcgctcgctcgctcactgaggccgcccgggcaaagcccgggcgtcgggcgacctttggtcgcccggcctcagtgagcgagcgagcgcgcagagagggagtggccaactccatcactaggggttccttgtagttaatgattaacccgccatgctacttatctacgtagccatgctctaggaagatcggaattcgcccttaagctagcagatcttccccacctagccacctggcaaactgctccttctctcaaaggcccaaacatggcctcccagactgcaacccccaggcagtcaggccctgtctccacaacctcacagccaccctggacggaatctgcttcttcccacatttgagtcctcctcagcccctgagctcctctgggcagggctgtttctttccatctttgtattcccaggggcctgcaaataaatgtttaatgaacgaacaagagagtgaattccaattccatgcaacaaggattgggctcctgggccctaggctatgtgtctggcaccagaaacggaagctgcaggttgcagcccctgccctcatggagctcctcctgtcagaggagtgtggggactggatgactccagaggtaacttgtgggggaacgaacaggtaaggggctgtgtgacgagatgagagactgggagaataaaccagaaagtctctagctgtccagaggacatagcacagaggcccatggtccctatttcaaacccaggccaccagactgagctgggaccttgggacagacaagtcatgcagaagttaggggaccttctcctcccttttcctggatggatcctgagtaccttctcctccctgacctcaggcttcctcctagtgtcaccttggcccctcttagaagccaattaggccctcagtttctgcagcggggattaatatgattatgaacacccccaatctcccagatgctgattcagccaggagcttaggagggggaggtcactttataagggtctgggggggtcagaacccagagtcatcccctgaattctgcagatatccatcacactggcggccgcgccaccatgtcacgcaagatagaaggctttttgttattacttctctttggctatgaagccacattgggattatcgtctaccgaggatgaaggcgaggacccctggtaccaaaaagcatgcaagtgcgattgccaaggaggacccaatgctctgtggtctgcaggtgccacctccttggactgtataccagaatgcccatatcacaagcctctgggtttcgagtcaggggaggtcacaccggaccagatcacctgctctaacccggagcagtatgtgggctggtattcttcgtggactgcaaacaaggcccggctcaacagtcaaggctttgggtgtgcctggctctccaagttccaggacagtagccagtggttacagatagatctgaaggagatcaaagtgatttcagggatcctcacccaggggcgctgtgacatcgatgagtggatgaccaagtacagcgtgcagtacaggaccgatgagcgcctgaactggatttactacaaggaccagactggaaacaaccgggtcttctatggcaactcggaccgcacctccacggttcagaacctgctgcggccccccatcatctcccgcttcatccgcctcatcccgctgggctggcacgtccgcattgccatccggatggagctgctggagtgcgtcagcaagtgtgcctgaa

SEQ ID NO: 19 - protein, 346 aa, Homo sapiens
MALLKVKFDQKKRVKLAQGLWLMNWFSVLAGIIIFSLGLFLKIELRKRSDVMNNSESHFVPNSLIGMGVLSCVFNSLAGKICYDALDPAKYARWKPWLKPYLAICVLFNIILFLVALCCFLLRGSLENTLGQGLKNGMKYYRDTDTPGRCFMKKTIDMLQIEFKCCGNNGFRDWFEIQWISNRYLDFSSKEVKDRIKSNVDGRYLVDGVPFSCCNPSSPRPCIQYQITNNSAHYSYDHQTEELNLWVRGCRAALLSYYSSLMNSMGVVTLLIWLFEVTITIGLRYLQTSLDGVSNPEESESESQGWLLERSVPETWKAFLESVKKLGKGNQVEAEGADAGQAPEAG

SEQ ID NO: 20 - protein, 470 aa, Homo sapiens
MSHHPSGLRAGFSSTSYRRTFGPPPSLSPGAFSYSSSSRFSSSRLLGSASPSSSVRLGSFRSPRAGAGALLRLPSERLDFSMAEALNQEFLATRSNEKQELQELNDRFANFIEKVRFLEQQNAALRGELSQARGQEPARADQLCQQELRELRRELELLGRERDRVQVERDGLAEDLAALKQRLEEETRKREDAEHNLVLFRKDVDDATLSRLELERKIESLMDEIEFLKKLHEEELRDLQVSVESQQVQQVEVEATVKPELTAALRDIRAQYESIAAKNLQEAEEWYKSKYADLSDAANRNHEALRQAKQEMNESRRQIQSLTCEVDGLRGTNEALLRQLRELEEQFALEAGGYQAGAARLEEELRQLKEEMARHLREYQELLNVKMALDIEIATYRKLLEGEESRISVPVHSFASLNIKTTVPEVEPPQDSHSRKTVLIKTIETRNGEVVTESQKEQRSELDKSSAHSY

SEQ ID NO: 21 - protein, 1286 aa, Homo sapiens
MSHLVDPTSGDLPVRDIDAIPLVLPASKGKNMKTQPPLSRMNREELEDSFFRLREDHMLVKELSWKQQDEIKRLRTTLLRLTAAGRDLRVAEEAAPLSETARRGQKAGWRQRLSMHQRPQMHRLQGHFHCVGPASPRRAQPRVQVGHRQLHTAGAPVPEKPKRGPRDRLSYTAPPSFKEHATNENRGEVASKPSELVSGSNSIISFSSVISMAKPIGLCMPNSAHIMASNTMQVEEPPKSPEKMWPKDENFEQRSSLECAQKAAELRASIKEKVELIRLKKLLHERNASLVMTKAQLTEVQEAYETLLQKNQGILSAAHEALLKQVNELRAELKEESKKAVSLKSQLEDVSILQMTLKEFQERVEDLEKERKLLNDNYDKLLESMLDSSDSSSQPHWSNELIAEQLQQQVSQLQDQLDAELEDKRKVLLELSREKAQNEDLKLEVTNILQKHKQEVELLQNAATISQPPDRQSEPATHPAVLQENTQIEPSEPKNQEEKKLSQVLNELQVSHAETTLELEKTRDMLILQRKINVCYQEELEAMMTKADNDNRDHKEKLERLTRLLDLKNNRIKQLEGILRSHDLPTSEQLKDVAYGTRPLSLCLETLPAHGDEDKVDISLLHQGENLFELHIHQAFLTSAALAQAGDTQPTTFCTYSFYDFETHCTPLSVGPQPLYDFTSQYVMETDSLFLHYLQEASARLDIHQAMASEHSTLAAGWICFDRVLETVEKVHGLATLIGAGGEEFGVLEYWMRLRFPIKPSLQACNKRKKAQVYLSTDVLGGRKAQEEEFRSESWEPQNELWIEITKCCGLRSRWLGTQPSPYAVYRFFTFSDHDTAIIPASNNPYFRDQARFPVLVTSDLDHYLRREALSIHVFDDEDLEPGSYLGRARVPLLPLAKNESIKGDFNLTDPAEKPNGSIQVQLDWKFPYIPPESFLKPEAQTKGKDTKDSSKISSEEEKASFPSQDQMASPEVPIEAGQYRSKRKPPHGGERKEKEHQVVSYSRRKHGKRIGVQGKNRMEYLSLNILNGNTPEQVNYTEWKFSETNSFIGDGFKNQHEEEEMTLSHSALKQKEPLHPVNDKESSEQGSEVSEAQTTDSDDVIVPPMSQKYPKADSEKMCIEIVSLAFYPEAEVMSDENIKQVYVEYKFYDLPLSETETPVSLRKPRAGEEIHFHFSKVIDLDPQEQQGRRRFLFDMLNGQDPDQGHLKFTVVSDPLDEEKKECEEVGYAYLQLWQILESGRDILEQELDIVSPEDLATPIGRLKVSLQAAAVLHAIYKEMTEDLFS

SEQ ID NO: 22 - protein, 240 aa, Adeno-associated virus-1
TFSYTFEEVPFHSSYAHSQSLDRLMNPLIDQYLYYLNRTQNQSGSAQNKDLLFSRGSPAGMSVQPKNWLPGPCYRQQRVSKTKTDNNNSNFTWTGASKYNLNGRESIINPGTAMASHKDDEDKFFPMSGVMIFGKESAGASNTALDNVMITDEEEIKATNPVATERFGTVAVNFQSSSTDPATGDVHAMGALPGMVWQDRDVYLQGPIWAKIPHTDGHFHPSPLMGGFGLKNPPPQILIK

SEQ ID NO: 23 - protein, 240 aa, Adeno-associated virus-6
TFSYTFEDVPFHSSYAHSQSLDRLMNPLIDQYLYYLNRTQNQSGSAQNKDLLFSRGSPAGMSVQPKNWLPGPCYRQQRVSKTKTDNNNSNFTWTGASKYNLNGRESIINPGTAMASHKDDKDKFFPMSGVMIFGKESAGASNTALDNVMITDEEEIKATNPVATERFGTVAVNLQSSSTDPATGDVHVMGALPGMVWQDRDVYLQGPIWAKIPHTDGHFHPSPLMGGFGLKHPPPQILIK

SEQ ID NO: 24 - protein, 240 aa, Adeno-associated virus-3
FSYTFEDVPFHSSYAHSQSLDRLMNPLIDQYLYYLNRTQGTTSGTTNQSRLLFSQAGPQSMSLQARNWLPGPCYRQQRLSKTANDNNNSNFPWTAASKYHLNGRDSLVNPGPAMASHKDDEEKFFPMHGNLIFGKEGTTASNAELDNVMITDEEEIRTTNPVATEQYGTVANNLQSSNTAPTTGTVNHQGALPGMVWQDRDVYLQGPIWAKIPHTDGHFHPSPLMGGFGLKHPPPQIMIK

SEQ ID NO: 25 - protein, 240 aa, Adeno-associated virus-2
FSYTFEDVPFHSSYAHSQSLDRLMNPLIDQYLYYLSRTNTPSGTTTQSRLQFSQAGASDIRDQSRNWLPGPCYRQQRVSKTSADNNNSEYSWTGATKYHLNGRDSLVNPGPAMASHKDDEEKFFPQSGVLIFGKQGSEKTNVDIEKVMITDEEEIRTTNPVATEQYGSVSTNLQRGNRQAATADVNTQGVLPGMVWQDRDVYLQGPIWAKIPHTDGHFHPSPLMGGFGLKHPPPQILIKN

SEQ ID NO: 26 - protein, 243 aa, Adeno-associated virus-8
NFQFTYTFEDVPFHSSYAHSQSLDRLMNPLIDQYLYYLSRTQTTGGTANTQTLGFSQGGPNTMANQAKNWLPGPCYRQQRVSTTTGQNNNSNFAWTAGTKYHLNGRNSLANPGIAMATHKDDEERFFPSNGILIFGKQNAARDNADYSDVMLTSEEEIKTTNPVATEEYGIVADNLQQQNTAPQIGTVNSQGALPGMVWQNRDVYLQGPIWAKIPHTDGNFHPSPLMGGFGLKHPPPQILIKN

SEQ ID NO: 27 - protein, 243 aa, synthetic construct
  REGION 1..243: note = Synthetic polypeptide
NFQFTYTFEDVPFHSSYAHSQSLDRLMNPLIDQYLYYLSRTQTTGGTANTQTLGFSQGGPNTMANQAKNWLPGPCYRQQRVSTTTGQNNNSNFAWTAGTKYHLNGRNSLANPGIAMATHKDDEERFFPSNGILIFGKQNAARDNADYSDVMLTSEEEIKTTNPVATEEYGIVADNLQGQRQAAQIGTVNSQGALPGMVWQNRDVYLQGPIWAKIPHTDGNFHPSPLMGGFGLKHPPPQILIKN

SEQ ID NO: 28 - protein, 241 aa, Adeno-associated virus-rh8
FQFSYTFEDVPFHSSYAHSQSLDRLMNPLIDQYLYYLVRTQTTGTGGTQTLAFSQAGPSSMANQARNWVPGPCYRQQRVSTTTNQNNNSNFAWTGAAKFKLNGRDSLMNPGVAMASHKDDDDRFFPSSGVLIFGKQGAGNDGVDYSQVLITDEEEIKATNPVATEEYGAVAINNQAANTQAQTGLVHNQGVIPGMVWQNRDVYLQGPIWAKIPHTDGNFHPSPLMGGFGLKHPPPQILIKN

SEQ ID NO: 29 - protein, 243 aa, Adeno-associated virus-10
NFEFSYTFEDVPFHSSYAHSQSLDRLMNPLIDQYLYYLSRTQSTGGTQGTQQLLFSQAGPANMSAQAKNWLPGPCYRQQRVSTTLSQNNNSNFAWTGATKYHLNGRDSLVNPGVAMATHKDDEERFFPSSGVLMFGKQGAGRDNVDYSSVMLTSEEEIKTTNPVATEQYGVVADNLQQANTGPIVGNVNSQGALPGMVWQNRDVYLQGPIWAKIPHTDGNFHPSPLMGGFGLKHPPPQILIKN

SEQ ID NO: 30 - protein, 242 aa, Adeno-associated virus-7
FEFSYSFEDVPFHSSYAHSQSLDRLMNPLIDQYLYYLARTQSNPGGTAGNRELQFYQGGPSTMAEQAKNWLPGPCFRQQRVSKTLDQNNNSNFAWTGATKYHLNGRNSLVNPGVAMATHKDDEDRFFPSSGVLIFGKTGATNKTTLENVLMTNEEEIRPTNPVATEEYGIVSSNLQAANTAAQTQVVNNQGALPGMVWQNRDVYLQGPIWAKIPHTDGNFHPSPLMGGFGLKHPPPQILIKN

SEQ ID NO: 31 - protein, 240 aa, Adeno-associated virus-9
FQFSYEFENVPFHSSYAHSQSLDRLMNPLIDQYLYYLSKTINGSGQNQQTLKFSVAGPSNMAVQGRNYIPGPSYRQQRVSTTVTQNNNSEFAWPGASSWALNGRNSLMNPGPAMASHKEGEDRFFPLSGSLIFGKQGTGRDNVDADKVMITNEEEIKTTNPVATESYGQVATNHQSAQAQAQTGWVQNQGILPGMVWQDRDVYLQGPIWAKIPHTDGNFHPSPLMGGFGMKHPPPQILIK

SEQ ID NO: 32 - protein, 239 aa, synthetic construct
  REGION 1..239: note = Synthetic polypeptide
QFSYEFENVPFHSSYAHSQSLDRLMNPLIDQYLYYLSKTINGSGQNQQTLKFSVAGPSNMAVQGRNYIPGPSYRQQRVSTTVTQNNNSEFAWPGASSWALNGRNSLMNPGPAMASHKEGEDRFFPLSGSLIFGKQGTGRDNVDADKVMITNEEEIKTTNPVATESYGQVATNHQSGQAQAATGWVQNQGILPGMVWQDRDVYLQGPIWAKIPHTDGNFHPSPLMGGFGMKHPPPQILIK

SEQ ID NO: 33 - protein, 240 aa, Adeno-associated virus-5
NFEFTYNFEEVPFHSSFAPSQNLFKLANPLVDQYLYRFVSTNNTGGVQFNKNLAGRYANTYKNWFPGPMGRTQGWNLGSGVNRASVSAFATTNRMELEGASYQVPPQPNGMTNNLQGSNTYALENTMIFNSQPANPGTTATYLEGNMLITSESETQPVNRVAYNVGGQMATNNQSSTTAPATGTYNLQEIVPGSVWMERDVYLQGPIWAKIPETGAHFHPSPAMGGFGLKHPPPMMLIKN

SEQ ID NO: 34 - protein, 250 aa, synthetic construct
  REGION 1..250: note = Synthetic polypeptide
TFSYTFEEVPFHSSYAHSQSLDRLMNPLIDQYLYYLNRTQNQSGSAQNKDLLFSRGSPAGMSVQPKNWLPGPCYRQQRVSKTKTDNNNSNFTWTGASKYNLNGRESIINPGTAMASHKDDEDKFFPMSGVMIFGKESAGASNTALDNVMITDEEEIKATNPVATERFGTVAVNFQSSSTDLALGETTRPAPATGDVHAMGALPGMVWQDRDVYLQGPIWAKIPHTDGHFHPSPLMGGFGLKNPPPQILIK

SEQ ID NO: 35 - protein, 250 aa, synthetic construct
  REGION 1..250: note = Synthetic polypeptide
TFSYTFEDVPFHSSYAHSQSLDRLMNPLIDQYLYYLNRTQNQSGSAQNKDLLFSRGSPAGMSVQPKNWLPGPCYRQQRVSKTKTDNNNSNFTWTGASKYNLNGRESIINPGTAMASHKDDKDKFFPMSGVMIFGKESAGASNTALDNVMITDEEEIKATNPVATERFGTVAVNLQSSSTDLALGETTRPAPATGDVHVMGALPGMVWQDRDVYLQGPIWAKIPHTDGHFHPSPLMGGFGLKHPPPQILIK

SEQ ID NO: 36 - protein, 250 aa, synthetic construct
  REGION 1..250: note = Synthetic polypeptide
FSYTFEDVPFHSSYAHSQSLDRLMNPLIDQYLYYLSRTNTPSGTTTQSRLQFSQAGASDIRDQSRNWLPGPCYRQQRVSKTSADNNNSEYSWTGATKYHLNGRDSLVNPGPAMASHKDDEEKFFPQSGVLIFGKQGSEKTNVDIEKVMITDEEEIRTTNPVATEQYGSVSTNLQRGNLALGETTRPARQAATADVNTQGVLPGMVWQDRDVYLQGPIWAKIPHTDGHFHPSPLMGGFGLKHPPPQILIKN

SEQ ID NO: 37 - protein, 253 aa, synthetic construct
  REGION 1..253: note = Synthetic polypeptide
NFQFTYTFEDVPFHSSYAHSQSLDRLMNPLIDQYLYYLSRTQTTGGTANTQTLGFSQGGPNTMANQAKNWLPGPCYRQQRVSTTTGQNNNSNFAWTAGTKYHLNGRNSLANPGIAMATHKDDEERFFPSNGILIFGKQNAARDNADYSDVMLTSEEEIKTTNPVATEEYGIVADNLQQQNLALGETTRPATAPQIGTVNSQGALPGMVWQNRDVYLQGPIWAKIPHTDGNFHPSPLMGGFGLKHPPPQILIKN

SEQ ID NO: 38 - protein, 252 aa, synthetic construct
  REGION 1..252: note = Synthetic polypeptide
NFQFTYTFEDVPFHSSYAHSQSLDRLMNPLIDQYLYYLSRTQTTGGTANTQTLGFSQGGPNTMANQAKNWLPGPCYRQQRVSTTTGQNNNSNFAWTAGTKYHLNGRNSLANPGIAMATHKDDEERFFPSNGILIFGKQNAARDNADYSDVMLTSEEEIKTTNPVATEEYGIVADNLQGQRGLGETTRPAQAAQIGTVNSQGALPGMVWQNRDVYLQGPIWAKIPHTDGNFHPSPLMGGFGLKHPPPQILIKN

SEQ ID NO: 39 - protein, 251 aa, synthetic construct
  REGION 1..251: note = Synthetic polypeptide
FQFSYTFEDVPFHSSYAHSQSLDRLMNPLIDQYLYYLVRTQTTGTGGTQTLAFSQAGPSSMANQARNWVPGPCYRQQRVSTTTNQNNNSNFAWTGAAKFKLNGRDSLMNPGVAMASHKDDDDRFFPSSGVLIFGKQGAGNDGVDYSQVLITDEEEIKATNPVATEEYGAVAINNQAANLALGETTRPATQAQTGLVHNQGVIPGMVWQNRDVYLQGPIWAKIPHTDGNFHPSPLMGGFGLKHPPPQILIKN

SEQ ID NO: 40 - protein, 253 aa, synthetic construct
  REGION 1..253: note = Synthetic polypeptide
NFEFSYTFEDVPFHSSYAHSQSLDRLMNPLIDQYLYYLSRTQSTGGTQGTQQLLFSQAGPANMSAQAKNWLPGPCYRQQRVSTTLSQNNNSNFAWTGATKYHLNGRDSLVNPGVAMATHKDDEERFFPSSGVLMFGKQGAGRDNVDYSSVMLTSEEEIKTTNPVATEQYGVVADNLQQLALGETTRPAANTGPIVGNVNSQGALPGMVWQNRDVYLQGPIWAKIPHTDGNFHPSPLMGGFGLKHPPPQILIKN

SEQ ID NO: 41 - protein, 252 aa, synthetic construct
  REGION 1..252: note = Synthetic polypeptide
FEFSYSFEDVPFHSSYAHSQSLDRLMNPLIDQYLYYLARTQSNPGGTAGNRELQFYQGGPSTMAEQAKNWLPGPCFRQQRVSKTLDQNNNSNFAWTGATKYHLNGRNSLVNPGVAMATHKDDEDRFFPSSGVLIFGKTGATNKTTLENVLMTNEEEIRPTNPVATEEYGIVSSNLQAANLALGETTRPATAAQTQVVNNQGALPGMVWQNRDVYLQGPIWAKIPHTDGNFHPSPLMGGFGLKHPPPQILIKN

SEQ ID NO: 42 - protein, 249 aa, synthetic construct
  REGION 1..249: note = Synthetic polypeptide
FQFSYEFENVPFHSSYAHSQSLDRLMNPLIDQYLYYLSKTINGSGQNQQTLKFSVAGPSNMAVQGRNYIPGPSYRQQRVSTTVTQNNNSEFAWPGASSWALNGRNSLMNPGPAMASHKEGEDRFFPLSGSLIFGKQGTGRDNVDADKVMITNEEEIKTTNPVATESYGQVATNHQSAQLALGETTRPAQAQTGWVQNQGILPGMVWQDRDVYLQGPIWAKIPHTDGNFHPSPLMGGFGMKHPPPQILIK

SEQ ID NO: 43 - protein, 248 aa, synthetic construct
  REGION 1..248: note = Synthetic polypeptide
QFSYEFENVPFHSSYAHSQSLDRLMNPLIDQYLYYLSKTINGSGQNQQTLKFSVAGPSNMAVQGRNYIPGPSYRQQRVSTTVTQNNNSEFAWPGASSWALNGRNSLMNPGPAMASHKEGEDRFFPLSGSLIFGKQGTGRDNVDADKVMITNEEEIKTTNPVATESYGQVATNHQSGQAALGETTRPAQAATGWVQNQGILPGMVWQDRDVYLQGPIWAKIPHTDGNFHPSPLMGGFGMKHPPPQILIK

SEQ ID NO: 44 - protein, 250 aa, synthetic construct
  REGION 1..250: note = Synthetic peptide
NFEFTYNFEEVPFHSSFAPSQNLFKLANPLVDQYLYRFVSTNNTGGVQFNKNLAGRYANTYKNWFPGPMGRTQGWNLGSGVNRASVSAFATTNRMELEGASYQVPPQPNGMTNNLQGSNTYALENTMIFNSQPANPGTTATYLEGNMLITSESETQPVNRVAYNVGGQMATNNQSLALGETTRPASTTAPATGTYNLQEIVPGSVWMERDVYLQGPIWAKIPETGAHFHPSPAMGGFGLKHPPPMMLIKN

SEQ ID NO: 45 - protein, 10 aa, synthetic construct
  REGION 1..10: note = Synthetic polypeptide
LALGETTRPA

SEQ ID NO: 46 - protein, 10 aa, synthetic construct
  REGION 1..10: note = Synthetic polypeptide
LANETITRPA

SEQ ID NO: 47 - protein, 10 aa, synthetic construct
  REGION 1..10: note = Synthetic polypeptide
LAKAGQANNA

SEQ ID NO: 48 - protein, 10 aa, synthetic construct
  REGION 1..10: note = Synthetic polypeptide
LAKDPKTTNA

SEQ ID NO: 49 - protein, 10 aa, synthetic construct
  REGION 1..10: note = Synthetic polypeptide
AALGETTRPA

SEQ ID NO: 50 - protein, 10 aa, synthetic construct
  REGION 1..10: note = Synthetic peptide
AANETITRPA

SEQ ID NO: 51 - protein, 10 aa, synthetic construct
  REGION 1..10: note = Synthetic polypeptide
AAKAGQANNA

SEQ ID NO: 52 - protein, 10 aa, synthetic construct
  REGION 1..10: note = Synthetic polypeptide
AAKDPKTTNA

SEQ ID NO: 53 - protein, 9 aa, synthetic construct
  REGION 1..9: note = Synthetic polypeptide
GLGETTRPA

SEQ ID NO: 54 - protein, 9 aa, synthetic construct
  REGION 1..9: note = Synthetic polypeptide
GNETITRPA

SEQ ID NO: 55 - protein, 9 aa, synthetic construct
  REGION 1..9: note = Synthetic polypeptide
GKAGQANNA

SEQ ID NO: 56 - protein, 9 aa, synthetic construct
  REGION 1..9: note = Synthetic peptide
GKDPKTTNA

SEQ ID NO: 57 - protein, 7 aa, synthetic construct
  REGION 1..7: note = Synthetic polypeptide
KDTDTTR

SEQ ID NO: 58 - protein, 7 aa, synthetic construct
  REGION 1..7: note = Synthetic polypeptide
RAGGSVG

SEQ ID NO: 59 - protein, 7 aa, synthetic construct
  REGION 1..7: note = Synthetic polypeptide
AVDTTKF

SEQ ID NO: 60 - protein, 7 aa, synthetic construct
  REGION 1..7: note = Synthetic polypeptide
STGKVPN

SEQ ID NO: 61 - protein, 10 aa, synthetic construct
  REGION 1..10: note = Synthetic polypeptide
LAKDTDTTRA

SEQ ID NO: 62 - protein, 10 aa, synthetic construct
  REGION 1..10: note = Synthetic polypeptide
LARAGGSVGA

SEQ ID NO: 63 - protein, 10 aa, synthetic construct
  REGION 1..10: note = Synthetic polypeptide
LAAVDTTKFA

SEQ ID NO: 64 - protein, 10 aa, synthetic construct
  REGION 1..10: note = Synthetic polypeptide
LASTGKVPNA